European Patent Application EP 4 653 009 A1, published November 26, 2025. Title: METHOD FOR TREATING SYSTEMIC LUPUS ERYTHEMATOSUS. Applicant: SHANGHAI HUAOTA BIOPHARMACEUTICAL CO., LTD. The sequence listing filed with the application follows.

SEQUENCE LISTING (39 sequences)

SEQ ID NO: 1 - protein, 12 aa, synthetic construct
  REGION 1..12: note = IL-36R antibody HCDR3
ARVDYGKPWFAY

SEQ ID NO: 2 - protein, 8 aa, synthetic construct
  REGION 1..8: note = IL-36R antibody HCDR2
IHPNSAKT

SEQ ID NO: 3 - protein, 8 aa, synthetic construct
  REGION 1..8: note = IL-36R antibody HCDR1
GYTFTSSW

SEQ ID NO: 4 - protein, 119 aa, synthetic construct
  REGION 1..119: note = IL-36R antibody VH
QVQLVQSGAEVKKPGASVKVSCKASGYTFTSSWMHWAKQAPGQGLEWIGEIHPNSAKTNYNQKFQGRVTMTRDTSISTAYMELSRLRSDDTAVYYCARVDYGKPWFAYWGQGTLVTVSS

SEQ ID NO: 5 - protein, 9 aa, synthetic construct
  REGION 1..9: note = IL-36R antibody LCDR3
QQFQSSPLT

SEQ ID NO: 6 - skipped

SEQ ID NO: 7 - protein, 7 aa, synthetic construct
  REGION 1..7: note = IL-36R antibody LCDR1
SSVSSSY

SEQ ID NO: 8 - protein, 108 aa, synthetic construct
  REGION 1..108: note = IL-36R antibody VL
QIVLTQSPGTLSLSPGERATLSCRASSSVSSSYLHWYQQKPGQAPRLWIYSTSSRATGIPDRFSGSGSGTDFTLTISRLEPEDFATYYCQQFQSSPLTFGQGTKLEIK

SEQ ID NO: 9 - protein, 329 aa, synthetic construct
  REGION 1..329: note = IL-36R antibody heavy chain constant region
ASTKGPSVFPLAPSSKSTSGGTAALGCLVKDYFPEPVTVSWNSGALTSGVHTFPAVLQSSGLYSLSSVVTVPSSSLGTQTYICNVNHKPSNTKVDKRVEPKSCDKTHTCPPCPAPEAAGGPSVFLFPPKPKDTLMISRTPEVTCVVVDVSHEDPEVKFNWYVDGVEVHNAKTKPREEQYNSTYRVVSVLTVLHQDWLNGKEYKCKVSNKALPAPIEKTISKAKGQPREPQVYTLPPSREEMTKNQVSLTCLVKGFYPSDIAVEWESNGQPENNYKTTPPVLDSDGSFFLYSKLTVDKSRWQQGNVFSCSVMHEALHNHYTQKSLSLSPG

SEQ ID NO: 10 - protein, 107 aa, synthetic construct [sequence omitted]

SEQ ID NO: 11 - protein, 448 aa, synthetic construct
  REGION 1..448: note = IL-36R antibody heavy chain
QVQLVQSGAEVKKPGASVKVSCKASGYTFTSSWMHWAKQAPGQGLEWIGEIHPNSAKTNYNQKFQGRVTMTRDTSISTAYMELSRLRSDDTAVYYCARVDYGKPWFAYWGQGTLVTVSSASTKGPSVFPLAPSSKSTSGGTAALGCLVKDYFPEPVTVSWNSGALTSGVHTFPAVLQSSGLYSLSSVVTVPSSSLGTQTYICNVNHKPSNTKVDKRVEPKSCDKTHTCPPCPAPEAAGGPSVFLFPPKPKDTLMISRTPEVTCVVVDVSHEDPEVKFNWYVDGVEVHNAKTKPREEQYNSTYRVVSVLTVLHQDWLNGKEYKCKVSNKALPAPIEKTISKAKGQPREPQVYTLPPSREEMTKNQVSLTCLVKGFYPSDIAVEWESNGQPENNYKTTPPVLDSDGSFFLYSKLTVDKSRWQQGNVFSCSVMHEALHNHYTQKSLSLSPG

SEQ ID NO: 12 - protein, 215 aa, synthetic construct
  REGION 1..215: note = IL-36R antibody light chain
QIVLTQSPGTLSLSPGERATLSCRASSSVSSSYLHWYQQKPGQAPRLWIYSTSSRATGIPDRFSGSGSGTDFTLTISRLEPEDFATYYCQQFQSSPLTFGQGTKLEIKRTVAAPSVFIFPPSDEQLKSGTASVVCLLNNFYPREAKVQWKVDNALQSGNSQESVTEQDSKDSTYSLSSTLTLSKADYEKHKVYACEVTHQGLSSPVTKSFNRGEC

SEQ ID NO: 13 - protein, 10 aa, synthetic construct
  REGION 1..10: note = IL-17A antibody HCDR3
ANYGWGYFDY

SEQ ID NO: 14 - protein, 8 aa, synthetic construct
  REGION 1..8: note = IL-17A antibody HCDR2
IDTNTGEP

SEQ ID NO: 15 - protein, 8 aa, synthetic construct
  REGION 1..8: note = IL-17A antibody HCDR1
EYIFTNYG

SEQ ID NO: 16 - protein, 117 aa, synthetic construct
  REGION 1..117: note = IL-17A antibody VH
QVQLVQSGSELKKPGASVKVSCKASEYIFTNYGMNWVKQAPGQGFEWMGWIDTNTGEPTYAQGFTGRFVFSLDTSVSTAYLQISSLKAEDTATYYCANYGWGYFDYWGQGTTVTVSS

SEQ ID NO: 17 - protein, 9 aa, synthetic construct
  REGION 1..9: note = IL-17A antibody LCDR3
SQSTHVPYT

SEQ ID NO: 18 - skipped

SEQ ID NO: 19 - protein, 11 aa, synthetic construct
  REGION 1..11: note = IL-17A antibody LCDR1
QSLVHSNGYTY

SEQ ID NO: 20 - protein, 112 aa, synthetic construct
  REGION 1..112: note = IL-17A antibody VL
DVVMTQTPPSLPVNPGEPASISCRSSQSLVHSNGYTYLHWYLQKPGQSPQLLIYKVSNHLSGVPDRFSGSGSGTDFTLKISWVEAEDVGVYFCSQSTHVPYTFGGGTKLEIK

SEQ ID NO: 21 - protein, 330 aa, synthetic construct
  REGION 1..330: note = IL-17A antibody heavy chain constant region
ASTKGPSVFPLAPSSKSTSGGTAALGCLVKDYFPEPVTVSWNSGALTSGVHTFPAVLQSSGLYSLSSVVTVPSSSLGTQTYICNVNHKPSNTKVDKRVEPKSCDKTHTCPPCPAPEAAGGPSVFLFPPKPKDTLMISRTPEVTCVVVDVSHEDPEVKFNWYVDGVEVHNAKTKPREEQYNSTYRVVSVLTVLHQDWLNGKEYKCKVSNKALPAPIEKTISKAKGQPREPQVYTLPPSREEMTKNQVSLTCLVKGFYPSDIAVEWESNGQPENNYKTTPPVLDSDGSFFLYSKLTVDKSRWQQGNVFSCSVMHEALHNHYTQKSLSLSPGK

SEQ ID NO: 22 - protein, 447 aa, synthetic construct
  REGION 1..447: note = IL-17A antibody heavy chain
QVQLVQSGSELKKPGASVKVSCKASEYIFTNYGMNWVKQAPGQGFEWMGWIDTNTGEPTYAQGFTGRFVFSLDTSVSTAYLQISSLKAEDTATYYCANYGWGYFDYWGQGTTVTVSSASTKGPSVFPLAPSSKSTSGGTAALGCLVKDYFPEPVTVSWNSGALTSGVHTFPAVLQSSGLYSLSSVVTVPSSSLGTQTYICNVNHKPSNTKVDKRVEPKSCDKTHTCPPCPAPEAAGGPSVFLFPPKPKDTLMISRTPEVTCVVVDVSHEDPEVKFNWYVDGVEVHNAKTKPREEQYNSTYRVVSVLTVLHQDWLNGKEYKCKVSNKALPAPIEKTISKAKGQPREPQVYTLPPSREEMTKNQVSLTCLVKGFYPSDIAVEWESNGQPENNYKTTPPVLDSDGSFFLYSKLTVDKSRWQQGNVFSCSVMHEALHNHYTQKSLSLSPGK

SEQ ID NO: 23 - protein, 219 aa, synthetic construct
  REGION 1..219: note = IL-17A antibody light chain; Bispecific antibody L chain
DVVMTQTPPSLPVNPGEPASISCRSSQSLVHSNGYTYLHWYLQKPGQSPQLLIYKVSNHLSGVPDRFSGSGSGTDFTLKISWVEAEDVGVYFCSQSTHVPYTFGGGTKLEIKRTVAAPSVFIFPPSDEQLKSGTASVVCLLNNFYPREAKVQWKVDNALQSGNSQESVTEQDSKDSTYSLSSTLTLSKADYEKHKVYACEVTHQGLSSPVTKSFNRGEC

SEQ ID NO: 24 - protein, 252 aa, synthetic construct
  REGION 1..252: note = IL-36R scFv
QIVLTQSPGTLSLSPGERATLSCRASSSVSSSYLHWYQQKPGQAPRLWIYSTSSRATGIPDRFSGSGSGTDFTLTISRLEPEDFATYYCQQFQSSPLTFGQGTKLEIKGGGGSGGGGSGGGGSGGGGSGGGGSQVQLVQSGAEVKKPGASVKVSCKASGYTFTSSWMHWAKQAPGQGLEWIGEIHPNSAKTNYNQKFQGRVTMTRDTSISTAYMELSRLRSDDTAVYYCARVDYGKPWFAYWGQGTLVTVSS

SEQ ID NO: 25 - protein, 718 aa, synthetic construct
  REGION 1..718: note = Bispecific antibody H chain
QVQLVQSGSELKKPGASVKVSCKASEYIFTNYGMNWVKQAPGQGFEWMGWIDTNTGEPTYAQGFTGRFVFSLDTSVSTAYLQISSLKAEDTATYYCANYGWGYFDYWGQGTTVTVSSASTKGPSVFPLAPSSKSTSGGTAALGCLVKDYFPEPVTVSWNSGALTSGVHTFPAVLQSSGLYSLSSVVTVPSSSLGTQTYICNVNHKPSNTKVDKRVEPKSCDKTHTCPPCPAPEAAGGPSVFLFPPKPKDTLMISRTPEVTCVVVDVSHEDPEVKFNWYVDGVEVHNAKTKPREEQYNSTYRVVSVLTVLHQDWLNGKEYKCKVSNKALPAPIEKTISKAKGQPREPQVYTLPPSREEMTKNQVSLTCLVKGFYPSDIAVEWESNGQPENNYKTTPPVLDSDGSFFLYSKLTVDKSRWQQGNVFSCSVMHEALHNHYTQKSLSLSPGGGGGSGGGGSGGGGSGGGGSQIVLTQSPGTLSLSPGERATLSCRASSSVSSSYLHWYQQKPGQAPRLWIYSTSSRATGIPDRFSGSGSGTDFTLTISRLEPEDFATYYCQQFQSSPLTFGQGTKLEIKGGGGSGGGGSGGGGSGGGGSGGGGSQVQLVQSGAEVKKPGASVKVSCKASGYTFTSSWMHWAKQAPGQGLEWIGEIHPNSAKTNYNQKFQGRVTMTRDTSISTAYMELSRLRSDDTAVYYCARVDYGKPWFAYWGQGTLVTVSS

SEQ ID NO: 26 - protein, 20 aa, synthetic construct
  REGION 1..20: note = linker
GGGGSGGGGSGGGGSGGGGS

SEQ ID NO: 27 - protein, 13 aa, synthetic construct
  REGION 1..13: note = muIL-36R antibody HCDR3
TRQEIYYSNYFDY

SEQ ID NO: 28 - protein, 8 aa, synthetic construct
  REGION 1..8: note = muIL-36R antibody HCDR2
FNPNNGGT

SEQ ID NO: 29 - protein, 8 aa, synthetic construct
  REGION 1..8: note = muIL-36R antibody HCDR1
GYTFTDYN

SEQ ID NO: 30 - protein, 120 aa, synthetic construct
  REGION 1..120: note = muIL-36R antibody VH
EVQLQQSGPELVKPGASVKMSCKASGYTFTDYNMHWVKQSHGKSLEWIGFFNPNNGGTRYNQKFKGKATLTVQKSSSTAYMDLRSLTSEDSAVYYCTRQEIYYSNYFDYWGQGTTLTVSS

SEQ ID NO: 31 - protein, 9 aa, synthetic construct
  REGION 1..9: note = muIL-36R antibody LCDR3
QQSYEDPYT

SEQ ID NO: 32 - skipped

SEQ ID NO: 33 - protein, 10 aa, synthetic construct
  REGION 1..10: note = muIL-36R antibody LCDR1
QSVDYDGDSY

SEQ ID NO: 34 - protein, 111 aa, synthetic construct
  REGION 1..111: note = muIL-36R antibody VL; 44G8 VL
DIVLTQSPASLAVSLGQRATISCKASQSVDYDGDSYMNWYQQKPGQPPKLLIYAASNLESGIPARFSGSGSGTDFTLNIHPVEEEDAATYSCQQSYEDPYTFGGGAKLEIK

SEQ ID NO: 35 - protein, 329 aa, synthetic construct
  REGION 1..329: note = muIL-36R antibody heavy chain constant region
AKTTAPSVYPLAPVCGDTTGSSVTLGCLVKGYFPEPVTLTWNSGSLSSGVHTFPAVLQSDLYTLSSSVTVTSSTWPSQSITCNVAHPASSTKVDKKIEPRGPTIKPCPPCKCPAPNLLGGPSVFIFPPKIKDVLMISLSPIVTCVVVAVSEDDPDVQISWFVNNVEVHTAQTQTHREDYASTLRVVSALPIQHQDWMSGKEFKCKVNNKDLPAPIERTISKPKGSVRAPQVYVLPPPEEEMTKKQVTLTCMVTDFMPEDIYVEWTNNGKTELNYKNTEPVLDSDGSYFMYSKLRVEKKNWVERNSYSCSVVHEGLHNHHTTKSFSRTPG

SEQ ID NO: 36 - protein, 107 aa, synthetic construct
  REGION 1..107: note = muIL-36R antibody lightchain constant region
RADAAPTVSIFPPSSEQLTSGGASVVCFLNNFYPKDINVKWKIDGSERQNGVLNSWTDQDSKDSTYSMSSTLTLTKDEYERHNSYTCEATHKTSTSPIVKSFNRNEC

SEQ ID NO: 37 - protein, 449 aa, synthetic construct
  REGION 1..449: note = muIL-36R antibody heavy chain
EVQLQQSGPELVKPGASVKMSCKASGYTFTDYNMHWVKQSHGKSLEWIGFFNPNNGGTRYNQKFKGKATLTVQKSSSTAYMDLRSLTSEDSAVYYCTRQEIYYSNYFDYWGQGTTLTVSSAKTTAPSVYPLAPVCGDTTGSSVTLGCLVKGYFPEPVTLTWNSGSLSSGVHTFPAVLQSDLYTLSSSVTVTSSTWPSQSITCNVAHPASSTKVDKKIEPRGPTIKPCPPCKCPAPNLLGGPSVFIFPPKIKDVLMISLSPIVTCVVVAVSEDDPDVQISWFVNNVEVHTAQTQTHREDYASTLRVVSALPIQHQDWMSGKEFKCKVNNKDLPAPIERTISKPKGSVRAPQVYVLPPPEEEMTKKQVTLTCMVTDFMPEDIYVEWTNNGKTELNYKNTEPVLDSDGSYFMYSKLRVEKKNWVERNSYSCSVVHEGLHNHHTTKSFSRTPG

SEQ ID NO: 38 - protein, 218 aa, synthetic construct
  REGION 1..218: note = muIL-36R antibody light chain
DIVLTQSPASLAVSLGQRATISCKASQSVDYDGDSYMNWYQQKPGQPPKLLIYAASNLESGIPARFSGSGSGTDFTLNIHPVEEEDAATYSCQQSYEDPYTFGGGAKLEIKRADAAPTVSIFPPSSEQLTSGGASVVCFLNNFYPKDINVKWKIDGSERQNGVLNSWTDQDSKDSTYSMSSTLTLTKDEYERHNSYTCEATHKTSTSPIVKSFNRNEC

SEQ ID NO: 39 - protein, 120 aa, synthetic construct
  REGION 1..120: note = 44G8 VH
EVQLQQSGPELVKPGASVKMSCKASGYTFTDYNMHWVKQSHGKSLEWIGFFNPNNGGTRYNQKFKGKATLTVNKSSSTAYMDLRSLTSEDSAVYYCTRQEIYYSNYFDYWGQGTTLTVSS